European Patent Application EP 4 814 107 A1, published September 30, 2026. Title: Phenol-producing Hydrogenophilus bacterium transformant. Applicant: 株式会社ＣＯ２資源化研究所. The sequence listing filed with the application follows.

SEQUENCE LISTING (17 sequences)

SEQ ID NO: 1 - DNA, 5219 bp, synthetic construct
  source 1..5219: mol_type = other DNA
cccatcgactgcacggtgcaccaatgcttctggcgtcaggcagccatcggaagctgtggtatggctgtgcaggtcgtaaatcactgcataattcgtgtcgctcaaggcgcactcccgttctggataatgttttttgcgccgacatcataacggttctggcaaatattctgaaatgagctgttgacaattaatcatcggctcgtataatgtgtggaattgtgagcggataacaatttcacacaggaaacaggccagttaggcctgctagcagatctggaggagaaacgcatatgctgatatcggatccgaattcgagctccgtcgacaagcttgcggccgcactgcagcaccatcaccaccatcattgataagatccggctgctaacaaagcccgaaaggaagctgagttggctgctgccaccgctgagcaataactcgaggccaatgaggccttcaaataaaacgaaaggctcagtcgaaagactgggcctttcgttttatctgttgtttgtcggtgaacgctctcctgagtaggacaaatccgccgggagcggatttgaacgttgcgaagcaacggcccggagggtggcgggcaggacgcccgccataaactgccaggcatcaaattaagcagaaggccatcctgacggatggcctttttgcgtttctacaaactccgcggatctaggtgaagatcctttttgataatctcatgaccaaaatcccttaacgtgagttttcgttccactgagcgtcagaccccgtagaaaagatcaaaggatcttcttgagatcctttttttctgcgcgtaatctgctgcttgcaaacaaaaaaaccaccgctaccagcggtggtttgtttgccggatcaagagctaccaactctttttccgaaggtaactggcttcagcagagcgcagataccaaatactgtccttctagtgtagccgtagttaggccaccacttcaagaactctgtagcaccgcctacatacctcgctctgctaatcctgttaccagtggctgctgccagtggcgataagtcgtgtcttaccgggttggactcaagacgatagttaccggataaggcgcagcggtcgggctgaacggggggttcgtgcacacagcccagcttggagcgaacgacctacaccgaactgagatacctacagcgtgagctatgagaaagcgccacgcttcccgaagggagaaaggcggacaggtatccggtaagcggcagggtcggaacaggagagcgcacgagggagcttccagggggaaacgcctggtatctttatagtcctgtcgggtttcgccacctctgacttgagcgtcgatttttgtgatgctcgtcaggggggcggagcctatggaaaaacgccagcaacgcggcctttttacggttcctggccttttgctggccgcggacgtagaaagccagtccgcagaaacggtgctgaccccggatgaatgtcagctactgggctatctggacaagggaaaacgcaagcgcaaagagaaagcaggtagcttgcagtgggcttacatggcgatagctagactgggcggttttatggacagcaagcgaaccggaattgccagctggggcgccctctggtaaggttgggaagccctgcaaagtaaactggatggctttcttgccgccaaggatctgatggcgcaggggatcaagatccgatcaagagaggccactaaggcccaggatgaggatcgtttcgcatgattgaacaagatggattgcacgcaggttctccggccgcttgggtggagaggctattcggctatgactgggcacaacagacaatcggctgctctgatgccgccgtgttccggctgtcagcgcaggggcgcccggttctttttgtcaagaccgacctgtccggtgccctgaatgaactacaggacgaggcagcgcggctatcgtggctggccacgacgggcgttccttgcgcagctgtgctcgacgttgtcactgaagcgggaagggactggctgctattgggcgaagtgccggggcaggatctcctgtcatctcaccttgctcctgccgagaaagtatccatcatggctgatgcaatgcggcggctgcatacgcttgatccggctacctgcccattcgaccaccaagcgaaacatcgcatcgagcgagcacgtactcggatggaagccggtcttgtcgatcaggatgatctggacgaagagcatcaggggctcgcgccagccgaactgttcgccaggctcaaggcgcgtatgcccgacggcgaggatctcgtcgtgactcatggcgatgcctgcttgccgaatatcatggtggaaaatggccgcttttctggattcatcgactgtggccggctgggtgtggcggaccgctatcaggacatagcgttggctacccgtgatattgctgaagagcttggcggcgaatgggctgaccgcttcctcgtgctttacggtatcgccgctcccgattcgcagcgcatcgccttctatcgccttcttgacgagttcttctgaggccatctaggccatgagtaagtctgacggaacggaaagttgtcggttaccagcaacgtttcgccctgttggcctcaaaagttcgagtccgttattggtatttccataccaactcaaacgggatataatgtgacatgtaacatttctcgattgaggaacgacaatgacagtaccggtcaaagcgcgtgttcaaaagtatcgcgacgcgctgcgccgctcgggtttgcgtccggttcagatatgggtgccggatacccgccgcccgggctttgcacaagagtgtcgccgccagtgcctgctcgtgacccaggcagacgccgctgatacgcaactccaacgactcatggatgaagccttggcagagattgatggctggcaggcatgatgcgcggcgatttggtaacgatcgttacccagggcgactttggcaaaccaaggccagcgttggtgatccagtccgatctgttcaacgagctcagcagcataaccgtctttcctgtaaccagtaccattgtggatgccccgttgttgcgcgtcacggttgagccaaccccggaaaacggcttgcacaagcgatcacaggtgatggtggacaaaattatgaccgtgcggcgggacaaagtcggtcagatcattggacgtatcgatacgactacgctgacaacgatcgagcgctgcttagctgtcttcttgggaatcgcgaaataaggccatgaaggccttacccatcaccgtgcatcacgccgaccgcttcgccactttgcgacaagaaagcaatctgaacgcgctggcgaaaatggatcggcgctgcccggtctacctgtgaagttcgcgcaaacgtccatcgagacgtacattgccgttggcatcgatctcgacggcgatttcctctggctaccgatcgcgcgcaccgcttacgcgccctcgacgtagtcgagaaaagcgtgattgcgtatgttgcgccaactgagcccgtcggtgcgttgtgaccactcgttgtagaccacgcccaaaaccatcaccccaaacggtgcggaaagtgctactctttcgtcttgccacaacaagaaggagggcgggtggtgatcgaaaccggtgctttgagagccaaagaagaccccattgcctgggtccaacagaaagcagccgaggcgttgcaacgcctagatcaaaagatggcctctcagcccgtgcagatgtacctaccggggttcgatctaggggcctttcccaaccatgtgaaccgctcctcgctctttgcgcctattgcgcgcggtcgccgcaaatttcatcgacaaacgaagatggtcagccgctcggatgctgtgatcgaatacactggagagcagctcgacgaagccgactgcgacctcatgatggcgctcatctggtttgcccagaaaaaaccgttaggggagtgggtgacattgaaccgagcgcagctgttgcggcggatcgggcgcgcgacgggcaagcagaactacgagtggctccatcgcagaatgcgggcgatgaccgaagcgacactctacatcgaagtgcgcaaatccgacggcagcacacgctacaagatcggctacgccgaggcgtttcacctcatcagcggctttgcgttcgatgagaaaagcgacgaatactgctaccaactcgatccccgctgggtacagctcttcagcaaccgcgaatacagcctgatcaacttcgacttgcgattgcagatcaaacggggtcaggacatggcgaaaaccctgcaacgcctcgttgctacttcttccgaccccatccagtcttacgaactcgaatggctcaagagcaaaatggaatacaccggaagaatgcgcgatttcaaagagtcgctctccaaggcgtgcaatgagctgaaacggttgcacatcgtcagtgaatacaagatcactctggacaaaaagaagcaacgggagctgttgaagctctggattcccaaagcgatcacggcataaaagcggtgcgacactgcacgatcagaaagtattttcagttactcaaacaccgttttttgttgaaaaacaacgaattgtcatcggtatagcgtcgcgcacccgagacgaccgacggtgtctggccatcggtatagcgtcgcgctttctccacctcttgaacagtcgttcggcatcggtatagcgtcgcgcctgcatcggtatagcgtcgcgctttttcggtatagcgtcgcgctttttcggtatagcgtcgcgcggttgtcaaaaaatctattattattcaataagttacaagcggtttttgaccgtctactatatttctacttatttctactaggaagcgcctgtggataacttcgctcttttctacacagcccctcagcggcgcaagcgcgccgctgggtagaaaattcctatcgcaacgaactgtcgttcctaaaaataggctactcggtaaaacaaccgtataaatgatgccgcgtgctcggagtcaactccagaacggcatcggtatagtgtcgcacttagcaatgtgcgaatatttcatcgttgagccgacttttggagattggtcatgggagatcctcgggttgtcgaagccttggactcctgttgatagatccagtaatgacctcagaactccatctggatttgttcagaacgctcggttgccgccgggcgttttttattggtgagaatccagtctaga

SEQ ID NO: 2 - DNA, 1425 bp, Chloroflexus aggregans
  source 1..1425: mol_type = genomic DNA
atggagatggaaccagacttcccacgcacgatgggtcagcagtttggccgccggtcgtgggccgagccgtggaagatcaagacggtcgagccgctgcggatcattagccgggccgagcgcgcggcagcgctgaaagccgccggctacaacacctttttactccgttcggaagatgtttatatcgatctgctcaccgatagcggcaccaatgctatgagcgaccggcagtgggcagcgttgatgatgggtgacgaggcgtatgccggtagccgcagtttctatcggttggaagcggcagtgcagcaggcttacggctatcgtcatgtcattcccacccaccaaggccgtggcgccgagcatctgatcagccggatcgctattcaacccggtcagtatgtgcccggtaatatgtatttcactactacccgtctccaccaagaactcgccggtggcatatttgttgatgtgattatcgatgaagctcacgatccgcagagccaatatcccttcaaggggaatgtcgatctcgataagctgcaaacgctgatcaatcaagttggcgcaaaacagattgcctacgtcagcctcgccggtacggtcaatatggccggcggccagccggtcagtatggcgaacgtgcgcgctttgcgcgaattgtgcgaccgctacggcatccgcatttttctcgacgcgacccggttggttgagaatgccttcttcatcaaagagcgcgaacccggctacgcgaatcatactatcgccgaaatcgtgcgcgagttttgtagctataccgacggtgcgtggatgagcgccaaaaaggatagtctggtcaacatcgggggctggctggcgctgaacgacgatcagcttgccgatgaggcgcgcaatctggtggtggtgtacgaggggttgcatacctacggcgggatggccgggcgcgatatggaagcattggcagttggaattgaggaatcattacaagaggactacattcgggcgcgaatcggccaagtgcgctaccttggcgaactgctgctcgattggaatatcccgattgtcgtgccgatcggtgggcacgcgattttcctcgatgctcgccgtttctacccacacctcccccaagacctcttccctgcccaaactttagccgctgagctgtacctcgattcgggggtacgggcaatggaacgtggtatcgccagtgccggacgcgatcctaagaccgggcagcaccactatcccaaactcgaactgacccgcctcaccatcccacgccgagtctatacccaagcccacatggacgtagttgccgaatcggtgaagtcggtctatgaccaacgtgaacgcgcccgtgggctgcgtatggtttatgagccgcgttacctgcgcttcttccaagcccgctttgaaccggttacggagtga

SEQ ID NO: 3 - protein, 474 aa, Chloroflexus aggregans
MEMEPDFPRTMGQQFGRRSWAEPWKIKTVEPLRIISRAERAAALKAAGYNTFLLRSEDVYIDLLTDSGTNAMSDRQWAALMMGDEAYAGSRSFYRLEAAVQQAYGYRHVIPTHQGRGAEHLISRIAIQPGQYVPGNMYFTTTRLHQELAGGIFVDVIIDEAHDPQSQYPFKGNVDLDKLQTLINQVGAKQIAYVSLAGTVNMAGGQPVSMANVRALRELCDRYGIRIFLDATRLVENAFFIKEREPGYANHTIAEIVREFCSYTDGAWMSAKKDSLVNIGGWLALNDDQLADEARNLVVVYEGLHTYGGMAGRDMEALAVGIEESLQEDYIRARIGQVRYLGELLLDWNIPIVVPIGGHAIFLDARRFYPHLPQDLFPAQTLAAELYLDSGVRAMERGIASAGRDPKTGQHHYPKLELTRLTIPRRVYTQAHMDVVAESVKSVYDQRERARGLRMVYEPRYLRFFQARFEPVTE

SEQ ID NO: 4 - DNA, 1419 bp, Chloroflexus aurantiacus
  source 1..1419: mol_type = genomic DNA
atgcaggaacaagactacccccgtacaatggggcaacaattcggtcggcggtcgtgggccgagccgtggaagatcaagatggttgagccgctgcgcgtgaccagccgggccgaacgcgaggcggcgctgaaggctgccggttacaacacgtttctgctgcgttctgaagatgtctatatcgatctgcttaccgatagtggtaccaatgccatgagcgaccggcaatgggcagccctgatgatgggcgacgaggcatacgccgggagccgcagtttttatcgcctggaagcaactgtccaacaggtgtatggctaccgccacattattcccacccatcaggggcggggcgccgagcatctgatcagtcaggtcgctatccgccgtgggcagtatgttcccggcaatatgtatttcacaaccacccgcctgcaccaggagctggccggtggcatctttgttgatgtgattattgacgaagcgcacgatccccaaagccagtatccgtttaaaggcaacgtcgatctcgacaaactacaggcgctgattgataaggttggcccgcaacagattgcctatatcagtctggccggtaccgtcaacatggctggtgggcagccggtcagtatggctaacgtccgtgccttacgcgcattatgtgatcggtacgggttgcgcatctttctcgattccacacgcttggttgagaatgcctttttcatcaaagaacgtgaacccggctatgccgaacaaagaatcgccgcgattgtccgcgagttttgcagttacaccgatggcgcatggatgagcgcaaagaaggacgcgctggtgaacatcggtggctggttagcgctcaacgatgatcaactcgccgatgaagcccgcaatctggtggtggtgtacgaagggttgcacacctacggcggcatggccgggcgtgatatggaggcgctggcggtcgggattgaggagtcgctgcaagaggattacatccgtgcccgcatcggtcaggtgcgctacctcggcgaactgctcctcgactgggacatccccatcgtagttccgattggcggtcacgcgatctttctggatgcacgccggttctatccgcacctgccgcaagacctcttccctgcccagaccctggccgccgagttgtacctcgattcaggggtgcgggctatggaacgcggtattgccagcgccggacgcgatcccaagaccgggcagaactactatcccaaactggaattaacccggctgaccatcccgcgccgtgtttatactcaggcccacatggatgttgtggccgagtcggtgaaggcagtgtacgatcaacgtcatcaggcccgtggcctgcggatggtctacgaaccacggtacctccgcttcttccaggcccggtttgaaccggtggaatga

SEQ ID NO: 5 - protein, 472 aa, Chloroflexus aurantiacus
MQEQDYPRTMGQQFGRRSWAEPWKIKMVEPLRVTSRAEREAALKAAGYNTFLLRSEDVYIDLLTDSGTNAMSDRQWAALMMGDEAYAGSRSFYRLEATVQQVYGYRHIIPTHQGRGAEHLISQVAIRRGQYVPGNMYFTTTRLHQELAGGIFVDVIIDEAHDPQSQYPFKGNVDLDKLQALIDKVGPQQIAYISLAGTVNMAGGQPVSMANVRALRALCDRYGLRIFLDSTRLVENAFFIKEREPGYAEQRIAAIVREFCSYTDGAWMSAKKDALVNIGGWLALNDDQLADEARNLVVVYEGLHTYGGMAGRDMEALAVGIEESLQEDYIRARIGQVRYLGELLLDWDIPIVVPIGGHAIFLDARRFYPHLPQDLFPAQTLAAELYLDSGVRAMERGIASAGRDPKTGQNYYPKLELTRLTIPRRVYTQAHMDVVAESVKAVYDQRHQARGLRMVYEPRYLRFFQARFEPVE

SEQ ID NO: 6 - DNA, 20 bp, synthetic construct
  source 1..20: mol_type = other DNA
gaattcgagctccgtcgaca

SEQ ID NO: 7 - DNA, 20 bp, synthetic construct
  source 1..20: mol_type = other DNA
atgcgtttctcctccagatc

SEQ ID NO: 8 - DNA, 1377 bp, Chryseobacterium gleum
  source 1..1377: mol_type = genomic DNA
atgaatttaccgtacgcggaacctttccgcatcaaaatggtggaagaaatctaccagtctaccagagaagaaagagagcagtggcttaaagaagctaattataaccttttcaatttaagatcttctcaggtttatattgacctgcttactgattccggaaccggagcaatgtccgataaacaatgggctgctttaatgacaggagatgaaagctacgcaggctcacgttcattcgaacaattacagaaaaccgttgaaagaattacaggattcaaatatttattaccaacccaccagggaagagccgctgaaaacgtgcttttttccgtattggtaaaagaaggtgatgtagttccgggaaactcacactttgacactacaaaaggtcatatcgagttcagaaaggcacatgcaatagattgtacgattgatgaagcttttgacatcaatgaccttcatcctttcaaagggaatatcaaccttgaaaaactggaagaagtttataaaagtcatcctaaagaaagtattcctttctgtctgattaccattacctgtaactcatcaggaggacagcctgtttctctggaaaatatgaaagctgtgaaagccctttctgatcaatatggaattcctgtattctttgattcagcgagatttgcagagaacgcctatttcatcaaaaaaagagaggcaggacaggaaaacagaagcattaaagacatctgtaaggaaattttctcttacggagacggaatgacaatgagttccaaaaaagacgggctggtaaacattggtggattcatcgctttgaataatgaagaagtgttcagaaaggcatccaactttaccattatctacgaaggctttattacttatggtggaatggccggaagagatatggcagcactggctgtaggtctggacgaagcgactgagtttgcttatcttgaaagcagaatctcccaggttgaatatcttgggaataaactgatcgaatatggaattcctgttcagaaaccaatcgggggacacgccgtatttattgattctttaaatttccttccgaatgtttcccgtgaagaatatccagcgcagacacttggtcttgaaatttataaagaagcaggaatcagaactgtagaaatcgggactttattagcagacagagatcctgcaacaagggaaaaccgttacccgaaattagaactggtacgtctcgcaattccaagaagaacttacaccaataatcatatggattatattgctgctgctataaagaacgtttatgaaagacgtgaagagattgcaaaagggtataagatcacctgggaacccgaaatcttaagacattttactgttcagcttgaaaaagcctaa

SEQ ID NO: 9 - DNA, 1371 bp, Serratia plymuthica
  source 1..1371: mol_type = genomic DNA
atgtcctacccagctgaaccttttcgcattaaaagcgttgaaaccctgacactgctttccaaagaggaaagagtaaaaaaaataatatctgcaggctataatacatttctattgaattcacgggatgtttatattgatctgctgacagacagcggcactaacgccatgagcgacaaacaatgggccggtataatgttgggtgatgaagcctatgccggcagtgaaaatttctttcatcttgaaagtaccgtacaagaattatttggtttccggtatctggtccccactcatcaggggcgtggcgcagaaaacctgctctctcaggtagcgattacccccgggcagtttgtcgccggcaatatgtacttcaccacaacccgctatcatcaggaaaaaaatggcgcggttttcgttgacgtcatcagagacgaagctcatgacgccagcgccattctgccgtttaaaggtgatattgacctgagcaagctagagacgctgatcgaggataaaggggcgaataacatcgcttatgtttgcctggcggtcaccgtcaatatggccggaggtcaaccggtctcgatgagtaacatgcgcgccgtccgcgcactgacccaacggcatggcatcaaagtctattacgatgcgacccgctgcgttgaaaacgcttacttcatcagagaaagagaagccggttacgaaaataccccgatttccgatatttttcatgaaatgtttagctatgccgacggctgcaccatgagcgggaaaaaagattgcctggtgaatatcggtggttttctgtgcatgaatgatgagaagctttttggcgccgtacgggagctggttgtcgtctatgaaggcatgccgtcctatggcggcctggcagggcgcgatatggaagcgatggccataggtctgcgtgaggcgatgcagtttgaatatattgagcatcgcgtcaagcaagtgcgttatttaggcgataaattgaaagccgccggcattcccattgttgaacccgtgggtggacatgccgttttcctggatgcccgacggttttgcccacatctgcaacaggagcaattgccggcacaaagcctcgccgccagcatttacgtagagactggagtacgcgccatggaacgcggtattgtctcctcggggcgcaataaggagaccggtgaaaactaccatcccaaacttgagacggtacgtctgacgataccgcgccgcgtatatacttacgcacatatggacagggtggccgatggcatcatcgaactgtttaaccggcgggaaaatatccgtggactgcgttttatttacgagcctaaacaactgcgcttctttaccgcgcgctttgaatatttgtga

SEQ ID NO: 10 - DNA, 42 bp, synthetic construct
  source 1..42: mol_type = other DNA
ctggaggagaaacgcatatggagatggaaccagacttcccac

SEQ ID NO: 11 - DNA, 44 bp, synthetic construct
  source 1..44: mol_type = other DNA
cgacggagctcgaattctcactccgtaaccggttcaaagcgggc

SEQ ID NO: 12 - DNA, 43 bp, synthetic construct
  source 1..43: mol_type = other DNA
ctggaggagaaacgcatatgcaggaacaagactacccccgtac

SEQ ID NO: 13 - DNA, 44 bp, synthetic construct
  source 1..44: mol_type = other DNA
cgacggagctcgaattctcattccaccggttcaaaccgggcctg

SEQ ID NO: 14 - DNA, 39 bp, synthetic construct
  source 1..39: mol_type = other DNA
ctggaggagaaacgcatatgaatttaccgtacgcggaac

SEQ ID NO: 15 - DNA, 40 bp, synthetic construct
  source 1..40: mol_type = other DNA
cgacggagctcgaattcttaggctttttcaagctgaacag

SEQ ID NO: 16 - DNA, 37 bp, synthetic construct
  source 1..37: mol_type = other DNA
ctggaggagaaacgcatatgtcctacccagctgaacc

SEQ ID NO: 17 - DNA, 39 bp, synthetic construct
  source 1..39: mol_type = other DNA
cgacggagctcgaattctcacaaatattcaaagcgcgcg